European Patent Application EP 4 613 862 A1, published September 10, 2025. Title: 一种抗病相关蛋白RCR1及其编码基因与应用. Applicant: 中国科学院遗传与发育生物学研究所. The sequence listing filed with the application follows.

SEQUENCE LISTING (22 sequences)

SEQ ID NO: 1 - DNA, 447 bp, synthetic construct
  source 1..447: mol_type = other DNA
atggagactgtctccgccgttaaccaaacactccccatctccggcggtgaaccggtgaagttcacgacatactctgccgcagttcacaaagtccttgtcatggtcaacgccggaattctagggttactccagcttgtcagccaacagtcctctgttttggaaacacataaagccgcattcctttgtttctgtgttttcattctattctacgccgttcttcgcgtccgtgaagccatggacgtgcgcctacaacccggtttagtcccaaggctcattggacatgggagccatctcttcggtggtctagccgctcttgtgctcgtctccgtcgttagtaccgcgttttctattgtcctttttcttctctggtttatctggctctccgccgtcgtctacttagagacaaacaaacccagtgcctgtccacctcagttaccaccagtttaa

SEQ ID NO: 2 - protein, 148 aa, synthetic construct
METVSAVNQTLPISGGEPVKFTTYSAAVHKVLVMVNAGILGLLQLVSQQSSVLETHKAAFLCFCVFILFYAVLRVREAMDVRLQPGLVPRLIGHGSHLFGGLAALVLVSVVSTAFSIVLFLLWFIWLSAVVYLETNKPSACPPQLPPV

SEQ ID NO: 3 - DNA, 4800 bp, synthetic construct
  source 1..4800: mol_type = other DNA
gatctggtaatgcgctgattctatcgcactccattatcgctacaaaaacaaggacaatatcaacaagaagaacgaaccatatgccttgagagtttctcaattaattccaaaaactagggtttattaaagtcggttaaaaaacaacatgagctagttctatagcactctatcgcttaaagataaagaaaaacaacgacaaaataaaccaacaaagtcgaatcatatgccttgagagtttgttgagtatacttacaatcgagggaggaggaatgaagaacgtaactaaccgacggtcaagtgaatatggccggagatctagctttaaggtgagcaagtgatacctactatatagtttatatagtttttcataaagacctttacaaggataacatttacaaaaacatttaccattataattaaatacattagctttttaatatatttcttaattttattaattatacatagatatgttttctattttattgagaacaaaatcttctcaaaatctagttgtcaaattttcattcaacttttaattataaaaaataagaaatttaaaagtaacttgtattcaaaaatgtcaaattaacaaaaaaattgtggtctcacacattattttctaactgctattcttaaattcgcaactaatatttgcttaatcaaatttactttcattttgaaataattatattttatccaaaaaaaggactattgtaaaataaatcaagattttttaaactaatattataatatatcaagatatttttatataattccattaaaaatctataatccccatcaaaattgattctatcatttgattattatttattaagattatatatcttattatataaatcttagttttcaaatatgtaaggaatataatttaacatatattaagtactcaataaaatttagttgcaaatatttatgtgtttatgatatcaacatattcaactaaacaattaataaggaggtaacatgtgttttaaaaattgtatgaaatgtgaaagtttgctcactcatattttgatcatccagttccagctaaactaaagaagttaaggtcccataaccgagaagtttgtcaaaagtttttattagatatttttaaatttaagaaacagataaactttacatggatttatcaatatcttcagatactttagataagtccattgaccacggcaaaggattattttaaagtacgtgaaaaaacattaagaaacagaaacaaaaagaaaaatgaaaagtttcgggaatgtttggatatcaagtaaataaaatgaattcgaagccttctctctttagaacttcgagtttttcgtctgataacgatgtttacgtattattatgatcatctcgcggctgcggagaaggacataagctcgaataatttctgtagtttggtggatgcttccgttatgttatacgacgaagaacaccgtgatcttcttccaaagaaagtaaactccagatgccaagcgaagacaaagaaacaagaaaaagagagtgacaagagattcttccatctcttccctaaaaaaagaagaacttcggttgttactgtaagaaccctgaacaaaaccaacaaaatctttataggatttctatttcttcatcgctcctcgaccttaacacgatccccggtgattcttctgacccacgtaacgaacttcaagggctttattattcttcttcttcatcgtttcttggagattacaagatcactgctgattacaagatgaaaaacccacaaacccctccttcttcttcaactttacttgttgagtacaacaccgagatgacaaaccctaattctcagacaaacagcaagagaaagtgtagtgctaatggtagtgaatccagtccagagccgtctcttaatgcctttcaacaccctaattcgtaacgactttttgacgcctgttgagtcgagaatcctactagaagaagatgacacggagggagttggagcgactctagtggatccatgggaggtaaagtggggtgtttttttgaagaaacggaagatgaagaaagattcagggaaaggaagcttgaattacgctattatctgcggatggaacgatatcgttgaggctaacgtattggaaaaagtcgatgacatcagtatttggtcttgatcaagtgtggatgatcaaggaagtaagatcttgatcaaggaagtaagatcttgatcaattcacagataatcggacggtcaccatttcacaggtatgcttcttagaattctcctataaacgagagttgaaagatcatgtttagcaactgatacaaaattgacatcaattataatatgggcaattgacaaaaataacaccaaaaaaattttcttccaatattaacacaatatttctaaaatttcacaaatagcactataaacttcaattaaacttaactaaaatataagatagaaaataaaaatgagagcagacactaatctaatattaaattgaatcaaataattttaaatagtggaaatatatactctaaattgaaaataaagaactcaaatataatactacaaactaatatttaaataaaaaatctcttttaaatggtgaaaatatataccctaaattagaaataggaaacccaaatataaaaccataaactaatattaaaatgaatcaaaattttcttaaatgattgaaatatataccctaaattggatatagagaaaccaaatataatattttaaatttatttctaatttattttggttgaatagattttatataaaaattatggtattattgagaaataaattagtgataatatttttagaataaaagctttatagtaagccaagtagtgctatttttgaaagtttatgaagtgtgcgttattattgttcataaaatttattttagtgctatttttaagaatttctcttataataatcgatttaagtattttgattattaacatcagtcagtaataatcttatgcaaattatatgcatcaccaatatataaatcacttatttaagtgatgcaaaatttttttacattatttttttaactaatgcaaatatttataataaatgatgtaaaacaatttttttttttagtgaaagtgaaagtgaattgaaagtgaagactagaaaaatcttgatcgttgcacaagccgagccgatgacagtcccttacacatgtgtttttggagccgatgactgtcatttttagataagtgtggaaagtggcttctatgtttttggagccgatgactgtcatttttagataagtgtggaaagtggcttctattcaaggaaggaaagtcaagccgagtatgatcttgatcaattcacagataatcggacggtcaccatttcacaggtatgcttcttagatttcttcttagatgtcacaggtgacgatgacagtcccttacacatgtgtttttggagctcctcacaggtgacgatgacagtcccttacacaggtgacgatgacagtccctttctttttatttatctttttttttattattgtaagggcctcttagatttctcctataaaacgagagttagaaagatcaagaaaatggtgcacaaaaaaaaaaacgaaagatcaagaaaacaaaagagaataaaactgcaaagatacaaattatggagactgtctccgccgttaaccaaacactccccatctccggcggtgaaccggtgaagttcacgacatactctgccgcagttcacaaagtccttgtcatggtcaacgccggaattctagggttactccagcttgtcagccaacagtcctctgttttggaaacacataaagccgcattcctttgtttctgtgttttcattctattctacgccgttcttcgcgtccgtgaagccatggacgtgcgcctacaacccggtttagtcccaaggctcattggacatgggagccatctcttcggtggtctagccgctcttgtgctcgtctccgtcgttagtaccgcgttttctattgtcctttttcttctctggtttatctggctctccgccgtcgtctacttagagacaaacaaacccagtgcctgtccacctcagttaccaccagtttaacatcttgtggttttatgaatggatgagtgtgagatgaaggttaatgtagaataacaccggtgacgttataaacagaccaatccggtagagactgtatcttggtaactagatgatgtggaagaatattccaaatatatttagttgacgtgaaagaaacagcctataaatcgagaatgctttctatatatgacgatttaatatatatattttccttgtgtgtttttcatactactacatttctgcagtatgctttggttatattattttattggtgaaatttacgtttattgaactgattggttcatacaaaaaccaatgttggcttctaatgggatttgtgatgactaaatgattcagttcacttttctttattgtttaacaaagatgcggataatcaaaagaaaattaaacttaaaaaaaacgctttggtcggtttagtcgttaaactatatataaactctgcaagtgttcatctaaaacattcaaaaatataatgtaacaaaggtttaaaacacgtagttttctttcgttttacaggataattatctgtgcaaaatcacttaaatagagtaaaagataactataatttacctatgcaaaatgagaagtgtttgtagatctaatcaaaagggtatgaatcaaagaaaaagaaaaaaagatttatttatgaatgttcctcgcagtttcccagatcccaacacctagtttcc

SEQ ID NO: 4 - DNA, 1356 bp, synthetic construct
  source 1..1356: mol_type = other DNA
acatcatttcttcttagctttttttcttcttcttcgttcatacagtttttttttgtttatcagcttacattttcttgaaccgtagctttcgttttcttctttttaactttccattcggagtttttgtatcttgtttcatagtttgtcccaggattcgaatgattaggcatcgaaccttcaagaatttgattgaataaaacatcttcattcttaagatatgaagataatcttcaaaaggcccctgggaatctgaaagaagagaagcaggcccatttatatgggaaagaacaatagtatttcttatataggcccatttaagttgaaaacaatcttcaaaagtcccacatcgcttagataagaaaacgaagctgagtttatatacagctagagtcgaagtagtggtggagtaaccctagaattcgttttagagctagaaatagcaagttaaaataaggctagtccgttatcaacttgaaaaagtggcaccgagtcggtgcttttttttgcaaaattttccagatcgatttcttcttcctctgttcttcggcgttcaatttctggggttttctcttcgttttctgtaactgaaacctaaaatttgacctaaaaaaaatctcaaataatatgattcagtggttttgtacttttcagttagttgagttttgcagttccgatgagataaaccaatattaatccaaactactgcagcctgacagacaaatgaggatgcaaacaattttaaagtttatctaacgctagctgttttgtttcttctctctggtgcaccaacgacggcgttttctcaatcataaagaggcttgttttacttaaggccaataatgttgatggatcgaaagaagagggcttttaataaacgagcccgtttaagctgtaaacgatgtcaaaaacatcccacatcgttcagttgaaaatagaagctctgtttatatattggtagagtcgactaagagattggtttagtcccaaggctcattagagctagaaatagcaagttaaaataaggctagtccgttatcaacttgaaaaagtggcaccgagtcggtgcttttttttgcaaaattttccagatcgatttcttcttcctctgttcttcggcgttcaatttctggggttttctcttcgttttctgtaactgaaacctaaaatttgacctaaaaaaaatctcaaataatatgattcagtggttttgtacttttcagttagttgagttttgcagttccgatgagataaaccaataccatggttattctagaaagcttgtcgacaagggtgggcgcgccgacccagctttcttgtacaaagttggcattataagaaagcattgcttatcaattt

SEQ ID NO: 5 - DNA, 7288 bp, synthetic construct
  source 1..7288: mol_type = other DNA
cctaatccgatcgagtacaaaagtaatgtaggacttagtgactacattagttagttaaaactataatatcgactggacaataattatatgtttgttgctcctttggtcgagacagaaccagaagaaattgagatgtatgtagtgaaagagttggtgatagaactaatagtgattaatttgttcagagacagagttgtgtaaactatgaagataatgttggtggactgagaatgtataaatttaacagtggctatgtggttattcttttgattttctttaaaatttcatattaattgaagaaacaatatgtattttcaagaaaatcaaaagacacagacaacaaagttagtgattgagatggaaatgtcaaaccgtttaaaaataagaaaccacaaaataattaaagttttttctatttttgtcaactatagaatgaaaattttggtatttttatcgacataatctagagcatggattggtttttttttttctgggatgaactgttatttttattattcagaccaaatctgagaattatttacaaactagtaaccataatgaaaggcaaaaccatagtacatcccagcaagagatgccctagttagcagactccatgcttgtgaaacaaggatggccataagctcggagtcggaccgaggcaacctgtttagaatcgttttattatttctatcaaacgggcaaagtgacttgtcgagtaaaagattttcttttcaatgctctcatttctatgccaaacattctctctttcagttgtatttgtctaactcgaaaatcttcaggtatatattaagagaatttagcaaaagttaattggatagtatatataactgaatgtagcttagctttttagcgcagaaaaaggcaattttcatgagaatagaattcctacaataatgttcaatgaaacaaatggtcatgtgcccaccaagtccccagcttcagcttcatatcaatcaactataacttggcatatgtgagaaagctttgtggatgtaagaagctccatgattatatcggaagctttgtcgggtataggacaatctttgaaacttagagtgagtttttttagtactgctgaattctcaagaaagtaattcgctagattaatcccagtttcctctcttatattcaggtttttaatcttaacatattccagagtcgatgttaaacatcgaggcacacttgtaaggtcgatttgccctggcaccggttcctgcgaaaatatacaaacaaactgagtttacaatatatttcaacaatgttcttaggggtaacgggtatgcacttttagtatataggctgtaaacttttacttcaaaaaagttatgtaaagaattttactctaacataatagactgtcaagattaggcttttcagatttgggcagctctcaagaaaggctgtcaacaattgtaacgatgtactgaagaaagaagcctccaaatgtgacaagttatggaatgtgggaatctgcagtaccattttcgagtaatggtaaaggacctgcaaagtagaaagaaaatgttttcatggaaagttaaattgttacatatgcatcaaagagtatatgtatatatctatacctctagagtatcattagagatgatcatatgtcttacaccagaaataccggtgagaaagtcacggattatatctctcttacttaaatccaccggttccaaaggactagtgtcaacattgacattaaagtcagtgtcgaggtctattttgaccaaggaactcaaattctttaccacgatcccagcagacagatcatctctaaaactcatatacttgagtctcggggcatcgatctcaactgaaaaaactgtactatacattccccaatagaacgttaaacaaaagatcttcagagtttgagacctcacacgcaaaacagagtgagattcttcattatcaaaattaggaactctcatcatagtaaattcttcaaggacagggcatcctaagaggagcttctctgtaatcttcgacggaccatcgtcgtaataaacgttgttgagatgcatgatcttgagacaaggtaaagaaacaacaagctcttgatgcttcattatcccaacatttgcaagctttaaagaaaccaatgtcttgctcttataaatattcttaggcatgaattctttaataaagataagattcgtgctcccaacatctagatgttgaactccgcgatcaaccgcagtggcgatccactccaagaatctgttggtatatacagtgttaccgccaaagtttaccttgaagtattgcatgtataacccacgattaaactccatatatttgttcacaaccatctgggaggctattccattaggagggaagttacagttctttaagtccaatccgacaacctttagccagacaaactcccatctcttagataaaacgcttgtcttaatcgaatctttgatcccaaggtatgagactatcttagctaccaaatgatctggtaatgcgctgattctatcgcactccattatcgctacaaaaacaaggacaatatcaacaagaagaacgaaccatatgccttgagagtttctcaattaattccaaaaactagggtttattaaagtcggttaaaaaacaacatgagctagttctatagcactctatcgcttaaagataaagaaaaacaacgacaaaataaaccaacaaagtcgaatcatatgccttgagagtttgttgagtatacttacaatcgagggaggaggaatgaagaacgtaactaaccgacggtcaagtgaatatggccggagatctagctttaaggtgagcaagtgatacctactatatagtttatatagtttttcataaagacctttacaaggataacatttacaaaaacatttaccattataattaaatacattagctttttaatatatttcttaattttattaattatacatagatatgttttctattttattgagaacaaaatcttctcaaaatctagttgtcaaattttcattcaacttttaattataaaaaataagaaatttaaaagtaacttgtattcaaaaatgtcaaattaacaaaaaaattgtggtctcacacattattttctaactgctattcttaaattcgcaactaatatttgcttaatcaaatttactttcattttgaaataattatattttatccaaaaaaaggactattgtaaaataaatcaagattttttaaactaatattataatatatcaagatatttttatataattccattaaaaatctataatccccatcaaaattgattctatcatttgattattatttattaagattatatatcttattatataaatcttagttttcaaatatgtaaggaatataatttaacatatattaagtactcaataaaatttagttgcaaatatttatgtgtttatgatatcaacatattcaactaaacaattaataaggaggtaacatgtgttttaaaaattgtatgaaatgtgaaagtttgctcactcatattttgatcatccagttccagctaaactaaagaagttaaggtcccataaccgagaagtttgtcaaaagtttttattagatatttttaaatttaagaaacagataaactttacatggatttatcaatatcttcagatactttagataagtccattgaccacggcaaaggattattttaaagtacgtgaaaaaacattaagaaacagaaacaaaaagaaaaatgaaaagtttcgggaatgtttggatatcaagtaaataaaatgaattcgaagccttctctctttagaacttcgagtttttcgtctgataacgatgtttacgtattattatgatcatctcgcggctgcggagaaggacataagctcgaataatttctgtagtttggtggatgcttccgttatgttatacgacgaagaacaccgtgatcttcttccaaagaaagtaaactccagatgccaagcgaagacaaagaaacaagaaaaagagagtgacaagagattcttccatctcttccctaaaaaaagaagaacttcggttgttactgtaagaaccctgaacaaaaccaacaaaatctttataggatttctatttcttcatcgctcctcgaccttaacacgatccccggtgattcttctgacccacgtaacgaacttcaagggctttattattcttcttcttcatcgtttcttggagattacaagatcactgctgattacaagatgaaaaacccacaaacccctccttcttcttcaactttacttgttgagtacaacaccgagatgacaaaccctaattctcagacaaacagcaagagaaagtgtagtgctaatggtagtgaatccagtccagagccgtctcttaatgcctttcaacaccctaattcgtaacgactttttgacgcctgttgagtcgagaatcctactagaagaagatgacacggagggagttggagcgactctagtggatccatgggaggtaaagtggggtgtttttttgaagaaacggaagatgaagaaagattcagggaaaggaagcttgaattacgctattatctgcggatggaacgatatcgttgaggctaacgtattggaaaaagtcgatgacatcagtatttggtcttgatcaagtgtggatgatcaaggaagtaagatcttgatcaaggaagtaagatcttgatcaattcacagataatcggacggtcaccatttcacaggtatgcttcttagaattctcctataaacgagagttgaaagatcatgtttagcaactgatacaaaattgacatcaattataatatgggcaattgacaaaaataacaccaaaaaaattttcttccaatattaacacaatatttctaaaatttcacaaatagcactataaacttcaattaaacttaactaaaatataagatagaaaataaaaatgagagcagacactaatctaatattaaattgaatcaaataattttaaatagtggaaatatatactctaaattgaaaataaagaactcaaatataatactacaaactaatatttaaataaaaaatctcttttaaatggtgaaaatatataccctaaattagaaataggaaacccaaatataaaaccataaactaatattaaaatgaatcaaaattttcttaaatgattgaaatatataccctaaattggatatagagaaaccaaatataatattttaaatttatttctaatttattttggttgaatagattttatataaaaattatggtattattgagaaataaattagtgataatatttttagaataaaagctttatagtaagccaagtagtgctatttttgaaagtttatgaagtgtgcgttattattgttcataaaatttattttagtgctatttttaagaatttctcttataataatcgatttaagtattttgattattaacatcagtcagtaataatcttatgcaaattatatgcatcaccaatatataaatcacttatttaagtgatgcaaaatttttttacattatttttttaactaatgcaaatatttataataaatgatgtaaaacaatttttttttttagtgaaagtgaaagtgaattgaaagtgaagactagaaaaatcttgatcgttgcacaagccgagccgatgacagtcccttacacatgtgtttttggagccgatgactgtcatttttagataagtgtggaaagtggcttctatgtttttggagccgatgactgtcatttttagataagtgtggaaagtggcttctattcaaggaaggaaagtcaagccgagtatgatcttgatcaattcacagataatcggacggtcaccatttcacaggtatgcttcttagatttcttcttagatgtcacaggtgacgatgacagtcccttacacatgtgtttttggagctcctcacaggtgacgatgacagtcccttacacaggtgacgatgacagtccctttctttttatttatctttttttttattattgtaagggcctcttagatttctcctataaaacgagagttagaaagatcaagaaaatggtgcacaaaaaaaaaaacgaaagatcaagaaaacaaaagagaataaaactgcaaagatacaaattatggagactgtctccgccgttaaccaaacactccccatctccggcggtgaaccggtgaagttcacgacatactctgccgcagttcacaaagtccttgtcatggtcaacgccggaattctagggttactccagcttgtcagccaacagtcctctgttttggaaacacataaagccgcattcctttgtttctgtgttttcattctattctacgccgttcttcgcgtccgtgaagccatggacgtgcgcctacaacccggtttagtcccaaggctcattggacatgggagccatctcttcggtggtctagccgctcttgtgctcgtctccgtcgttagtaccgcgttttctattgtcctttttcttctctggtttatctggctctccgccgtcgtctacttagagacaaacaaacccagtgcctgtccacctcagttaccaccagtttaacatcttgtggttttatgaatggatgagtgtgagatgaaggttaatgtagaataacaccggtgacgttataaacagaccaatccggtagagactgtatcttggtaactagatgatgtggaagaatattccaaatatatttagttgacgtgaaagaaacagcctataaatcgagaatgctttctatatatgacgatttaatatatatattttccttgtgtgtttttcatactactacatttctgcagtatgctttggttatattattttattggtgaaatttacgtttattgaactgattggttcatacaaaaaccaatgttggcttctaatgggatttgtgatgactaaatgattcagttcacttttctttattgtttaacaaagatgcggataatcaaaagaaaattaaacttaaaaaaaacgctttggtcggtttagtcgttaaactatatataaactctgcaagtgttcatctaaaacattcaaaaatataatgtaacaaaggtttaaaacacgtagttttctttcgttttacaggataattatctgtgcaaaatcacttaaatagagtaaaagataactataatttacctatgcaaaatgagaagtgtttgtagatctaatcaaaagggtatgaatcaaagaaaaagaaaaaaagatttatttatgaatgttcctcgcagtttcccagatcccaacacctagtttcc

SEQ ID NO: 6 - DNA, 22 bp, synthetic construct
  source 1..22: mol_type = other DNA
tggagtaaccctagaattccgg

SEQ ID NO: 7 - DNA, 22 bp, synthetic construct
  source 1..22: mol_type = other DNA
gtttagtcccaaggctcattgg

SEQ ID NO: 8 - DNA, 39 bp, synthetic construct
  source 1..39: mol_type = other DNA
atatatggtctcgattgtggagtaaccctagaattcgtt

SEQ ID NO: 9 - DNA, 41 bp, synthetic construct
  source 1..41: mol_type = other DNA
tgtggagtaaccctagaattcgttttagagctagaaatagc

SEQ ID NO: 10 - DNA, 43 bp, synthetic construct
  source 1..43: mol_type = other DNA
aacatgagccttgggactaaaccaatctcttagtcgactctac

SEQ ID NO: 11 - DNA, 37 bp, synthetic construct
  source 1..37: mol_type = other DNA
attattggtctcgaaacatgagccttgggactaaacc

SEQ ID NO: 12 - DNA, 46 bp, synthetic construct
  source 1..46: mol_type = other DNA
cgaattccgaattcgagctcgatctggtaatgcgctgattctatcg

SEQ ID NO: 13 - DNA, 41 bp, synthetic construct
  source 1..41: mol_type = other DNA
ttcatttcgaaggtaccggaaactaggtgttgggatctggg

SEQ ID NO: 14 - DNA, 20 bp, synthetic construct
  source 1..20: mol_type = other DNA
atggagactgtctccgccgt

SEQ ID NO: 15 - DNA, 19 bp, synthetic construct
  source 1..19: mol_type = other DNA
ttaaactggtggtaactga

SEQ ID NO: 16 - DNA, 19 bp, synthetic construct
  source 1..19: mol_type = other DNA
atggagactgtctccgccg

SEQ ID NO: 17 - DNA, 21 bp, synthetic construct
  source 1..21: mol_type = other DNA
gtaggattctggtgtgtgcgc

SEQ ID NO: 18 - DNA, 22 bp, synthetic construct
  source 1..22: mol_type = other DNA
aactctcccgctatgtatgtcg

SEQ ID NO: 19 - DNA, 20 bp, synthetic construct
  source 1..20: mol_type = other DNA
aaccctcgtagattggcaca

SEQ ID NO: 20 - DNA, 18 bp, synthetic construct
  source 1..18: mol_type = other DNA
caccgactacctgatgaa

SEQ ID NO: 21 - DNA, 17 bp, synthetic construct
  source 1..17: mol_type = other DNA
cagcttctccttgatgt

SEQ ID NO: 22 - DNA, 40 bp, synthetic construct
  source 1..40: mol_type = other DNA
cgaattccgaattcgagctccctaatccgatcgagtacaa